European Patent Application EP 4 417 263 A2, published August 21, 2024. Title: CD3 BINDING ANTIBODIES. Applicant: TeneoOne, Inc. The sequence listing filed with the application follows.

SEQUENCE LISTING (48 sequences)

SEQ ID NO: 1 - protein, 123 aa, Homo sapiens
EVQLVESGGGLVQPGRSLRLSCAASGFTFDDYAMHWVRQAPGKGLEWVSGISWNSGSIGYADSVKGRFTISRDNAKNSLYLQMNSLRAEDTALYYCAKDSRGYGDYRLGGAYWGQGTLVTVSS

SEQ ID NO: 2 - protein, 123 aa, Homo sapiens
EVQLVESGGGLVKPGGSLRLSCAASGFTFDDYAMHWVRQAPGKGLEWVSGISWNSGSIGYADSVKGRFTISRDNAKNSLYLQMNSLRAEDTALYYCAKDSRGYGDYRLGGAYWGQGTLVTVSS

SEQ ID NO: 3 - protein, 123 aa, Homo sapiens
EVQLVESGGGLVQPGRSLRLSCAASGFTFDDYAMHWVRQAPGKGLEWVSGISWNSGSIGYADSVKGRFTISRDNAKKSLYLQMNSLRAEDTALYYCAKDSRGYGDYSRGGAYWGQGTLVTVSS

SEQ ID NO: 4 - protein, 123 aa, Homo sapiens
EVQLVESGGGLVQPGRSLRLSCAASGFTFDDYAMHWVRQAPGKGLEWVSGISWNSGSIGYADSVKGRFTISRDNAKNSLYLQMNSLRPEDTALYYCAKDSRGYGDYSLGGAYWGQGTLVTVSS

SEQ ID NO: 5 - protein, 123 aa, Homo sapiens
EVQLVESGGGLVQPGRSLRLSCAASGFTFDDYAMHWVRQAPGKGLEWVSGISWNSGSIGYADSVKGRFTISRDNAKNSLYLQMNSLRAEDTALYYCAKDSRGYGDYSLGGAYWGQGTLVTVSS

SEQ ID NO: 6 - protein, 123 aa, Homo sapiens
EVQLVESGGGLVQPGRSLRLSCAASGFTFANYAMHWVRQAPGKGLEWVSGISWNSGSIDYADSVKGRFTISRDNAKNSLYLQMNSLRAEDTALYYCAKDSRGYGDYSRGGAYWGQGTLVTVSS

SEQ ID NO: 7 - protein, 123 aa, Homo sapiens
EVQLVESGGGLVQPGRSLRLSCAASGFTFNNYAMHWVRQAPGKGLEWVSGISWNSGSIGYADSVKGRFTISRDNAKNSLYLQMNSLRGEDTALYYCAKDSRGYGDYSRGGAYWGQGTLVTVSS

SEQ ID NO: 8 - protein, 123 aa, Homo sapiens
EVQLVESGGGLVQPGGSLRLSCAASGFTFADYAMHWVRQAPGKGLEWVSGISWNSGSIGYADSVKGRFTISRDNAKNSLYLQMNSLRAEDTALYYCAKDSRGYGDYSRGGAYWGQGTLVTVSS

SEQ ID NO: 9 - protein, 123 aa, Homo sapiens
EVQLVESGGGLVQPGRSLRLSCAASGFTFDNYAMHWVRQAPGKGLEWVSGISWNSGSIGYADSVKGRFTISRDNAKKSLYLQMNSLRAEDTALYYCAKDSRGYGDYSRGGAYWGQGTLVTVSS

SEQ ID NO: 10 - protein, 123 aa, Homo sapiens
EVQLVESGGGLVQPGRSLRLSCAASGFTFDNYAMHWVRQAPGKGLEWVSGISWNSGSIGYADSVKGRFTISRDNAKNSLYLQMNSLRAEDTALYYCAKDSRGYGDYSRGGAYWGQGTLVTVSS

SEQ ID NO: 11 - protein, 123 aa, Homo sapiens
EVQLVESGGGLVQPGRSLRLSCAASGFTFDDYAMHWVRQAPGKGLEWVSGISWNSGSIGYADSVKGRFTISRDNAKNSLYLQMNSLRAEDTALYYCAKDSRGYGDYSRGGAYWGQGTLVTVSS

SEQ ID NO: 12 - protein, 123 aa, Homo sapiens
EVQLVESGGGLVQPGRSLRLSCAASGFTFDDYAMHWVRQAPGKGLEWVSGISWNSGSIGYADSVKGRFTISRDNAKNSLYLQMNSLRPEDTALYYCAKDSRGYGSYSRGGAYWGQGTLVTVSS

SEQ ID NO: 13 - protein, 123 aa, Homo sapiens
EVQLVESGGGLVQPGRSLRLSCAASGFTFHNYAMHWVRQAPGKGLEWVSGISWNSGSIGYADSVKGRFTISRDNAKNSLYLQMNSLRAEDTALYYCAKDSRGYGDYSLGGAYWGQGTLVTVSS

SEQ ID NO: 14 - protein, 123 aa, Homo sapiens
EVQLVESGGGLVQPGGSLRLSCAASGFTFDDYAMHWVRQAPGKGLEWVSGISWNSGSIGYADSVKGRFTISRDNAKNSLYLQMNSLRAEDTALYYCAKDSRGYGDYSRGGAYCGQGTLVTVSS

SEQ ID NO: 15 - protein, 123 aa, Homo sapiens
EVQLVESGGGLVQPGRSLRLSCAASGFTFDNYAMHWVRQAPGKGLEWVSGISWNSGSIGYADSVKGRFTISRDNAKKSLYLQMNSLRAEDTALYYCAKDSRGYGDYSLGGAYWGQGTLVTVSS

SEQ ID NO: 16 - protein, 123 aa, Homo sapiens
EVQLVESGGGLVQPGRSLRLSCAASGFTFDDYAMHWVRQAPGKGLEWVSGISWNSGSIGYADSVKGRFTISRDNAKKSLYLQMNSLRAEDTALYYCAKDSRGYGDYRLGGAYWGQGTLVTVSS

SEQ ID NO: 17 - protein, 123 aa, Homo sapiens
EVQLVESGGGLVQPGRSLRLSCEASGFTFDDYAMHWVRQAPGKGLEWVSGISWNSGSIGYADSVKGRFTISRDNAKNSLYLQMNSLRAEDTALYYCAKDSRGYGDYRLGGAYWGQGTLVTVSS

SEQ ID NO: 18 - protein, 123 aa, Homo sapiens
EVQLVESGGGLVQPGRSLRLSCAASGFTFDDYAMHWVRQAPGKGLEWVSGISWNSGSIGYADSVKGRFTISRDNAKNSLYLQMNSLRPEDTALYYCAKDSRGYGDYRLGGAYWGQGTLVTVSS

SEQ ID NO: 19 - protein, 107 aa, Homo sapiens
EIVMTQSPATLSVSPGERATLSCRASQSVSSNLAWYQQKPGQAPRLLIYGASTRATGIPARFSGSGSGTEFTLTISSLQSEDFAVYYCQQYNNWPWTFGQGTKVEIK

SEQ ID NO: 20 - protein, 243 aa, Homo sapiens
EVQLLESGGGLVQPGGSLRLSCAASGFTVSSYGMSWVRQAPGKGPEWVSGIRGSDGSTYYADSVKGRFTISRDNSKNTLYLQMNSLRAEDTAVYYCAKQGENDGPFDHRGQGTLVTVSSGGGGSEVQLLESGGGLVQPGGSLRLSCAASGFTVSSYGMSWVRQAPGKGPEWVSGIRGSDGSTYYADSVKGRFTISRDNSKNTLYLQMNSLRAEDTAVYYCAKQGENDGPFDHRGQGTLVTVSS

SEQ ID NO: 21 - protein, 119 aa, Homo sapiens
EVQLLESGGGLVQPGGSLRLSCAASGFTVSSYGMSWVRQAPGKGPEWVSGIRGSDGSTYYADSVKGRFTISRDNSKNTLYLQMNSLRAEDTAVYYCAKQGENDGPFDHRGQGTLVTVSS

SEQ ID NO: 22 - protein, 128 aa, Homo sapiens
QLQLQESGPGLVKPSQTLSLTCTVSGGSISSGGHYWSWIRQHPGKGLEWIGYIHYSGSTYYNPSLKSRVIISVDTSKNQFSLKLRSVTAADTAVYYCARWRHDIFAAYPYYYYGMDVWGQGTLVTVSS

SEQ ID NO: 23 - protein, 8 aa, synthetic construct
  VARIANT 5..6: note = MOD_RES - Xaa is any amino acid
  source 1..8: note = Description of Artificial Sequence: Synthetic peptide
GFTFXXYA

SEQ ID NO: 24 - protein, 8 aa, Homo sapiens
ISWNSGSI

SEQ ID NO: 25 - protein, 16 aa, synthetic construct
  VARIANT 9: note = MOD_RES - Xaa is any amino acid
  VARIANT 11..12: note = MOD_RES - Xaa is any amino acid
  source 1..16: note = Description of Artificial Sequence: Synthetic peptide
AKDSRGYGXYXXGGAY

SEQ ID NO: 26 - protein, 16 aa, synthetic construct
  VARIANT 11..12: note = MOD_RES - Xaa is any amino acid
  source 1..16: note = Description of Artificial Sequence: Synthetic peptide
AKDSRGYGDYXXGGAY

SEQ ID NO: 27 - protein, 5 aa, synthetic construct
  source 1..5: note = Description of Artificial Sequence: Synthetic peptide
TVAAP

SEQ ID NO: 28 - protein, 6 aa, synthetic construct
  source 1..6: note = Description of Artificial Sequence: Synthetic peptide
ASTKGP

SEQ ID NO: 29 - protein, 8 aa, Homo sapiens
GFTFDDYA

SEQ ID NO: 30 - protein, 8 aa, Homo sapiens
GFTFANYA

SEQ ID NO: 31 - protein, 8 aa, Homo sapiens
GFTFNNYA

SEQ ID NO: 32 - protein, 8 aa, Homo sapiens
GFTFADYA

SEQ ID NO: 33 - protein, 8 aa, Homo sapiens
GFTFDNYA

SEQ ID NO: 34 - protein, 8 aa, Homo sapiens
GFTFHNYA

SEQ ID NO: 35 - protein, 6 aa, Homo sapiens
QSVSSN

SEQ ID NO: 36 - protein, 8 aa, Homo sapiens
GFTVSSYG

SEQ ID NO: 37 - protein, 10 aa, Homo sapiens
GGSISSGGHY

SEQ ID NO: 38 - skipped

SEQ ID NO: 39 - protein, 8 aa, Homo sapiens
IRGSDGST

SEQ ID NO: 40 - protein, 7 aa, Homo sapiens
IHYSGST

SEQ ID NO: 41 - protein, 16 aa, Homo sapiens
AKDSRGYGDYRLGGAY

SEQ ID NO: 42 - protein, 16 aa, Homo sapiens
AKDSRGYGDYSRGGAY

SEQ ID NO: 43 - protein, 16 aa, Homo sapiens
AKDSRGYGDYSLGGAY

SEQ ID NO: 44 - protein, 16 aa, Homo sapiens
AKDSRGYGSYSRGGAY

SEQ ID NO: 45 - protein, 9 aa, Homo sapiens
QQYNNWPWT

SEQ ID NO: 46 - protein, 12 aa, Homo sapiens
AKQGENDGPFDH

SEQ ID NO: 47 - protein, 20 aa, Homo sapiens
ARWRHDIFAAYPYYYYGMDV

SEQ ID NO: 48 - protein, 16 aa, synthetic construct
  VARIANT 11: note = MOD_RES - Arg or Ser
  VARIANT 12: note = MOD_RES - Leu or Arg
  source 1..16: note = Description of Artificial Sequence: Synthetic peptide
AKDSRGYGDYXXGGAY